European Patent Application EP 4 578 869 A1, published July 2, 2025. Title: 一种用于有效递送核酸的分支链结构多肽载体及其变化形式. Applicant: 苏州慧疗生物医药科技有限公司. Application CN. The sequence listing filed with the application follows.

SEQUENCE LISTING (12 sequences)

SEQ ID NO: 1 - protein, 18 aa, Synthetic Construct
KLSLLSLCKKKLSLLSLC

SEQ ID NO: 2 - protein, 21 aa, Synthetic Construct
KLLALLACKKKSKKLLALLAC

SEQ ID NO: 3 - protein, 19 aa, Synthetic Construct
KLLACKKKDKKKDKKLLAC

SEQ ID NO: 4 - protein, 24 aa, Synthetic Construct
KLLAKKKRCKKLLAKKKRCKKLLA

SEQ ID NO: 5 - protein, 37 aa, Synthetic Construct
KLAALAALAALAALAACKKKKLAALAALAALAALAAC

SEQ ID NO: 6 - protein, 36 aa, Synthetic Construct
KLSALSALSALSACKKKKKKKKKLSALSALSALSAC

SEQ ID NO: 7 - protein, 37 aa, Synthetic Construct
KLAALAALAACKKKAKAKKKKAKAKKKLAALAALAAC

SEQ ID NO: 8 - protein, 48 aa, Synthetic Construct
KLAALAALAAKKKRKRRCKKLAALAALAAKKKRKRRCKKLAALAALAA

SEQ ID NO: 9 - protein, 49 aa, Synthetic Construct
KLAALAALAALAALAALAALAACKKKKLAALAALAALAALAALAALAAC

SEQ ID NO: 10 - protein, 64 aa, Synthetic Construct
KLAALAALAALAALAALAALAACKKKSKKSKKSKKSKKSKKKLAALAALAALAALAALAALAAC

SEQ ID NO: 11 - protein, 63 aa, Synthetic Construct
KLAALAALAALAALAACKKKDKDKDKDKDKDKKKDKDKDKDKDKDKKLAALAALAALAALAAC

SEQ ID NO: 12 - protein, 74 aa, Synthetic Construct
KLAALAALAALAALAAKKKSKKSKKSKCKKLAALAALAALAALAAKKKSKKSKKSKCKKLAALAALAALAALAA